European Patent Specification EP 4 100 416 B1, published July 16, 2025. Title: COMPOSITIONS AND METHODS FOR RAPID RNA-ADENYLATION AND RNA SEQUENCING. Applicant: Cornell University. The sequence listing filed with the application follows.

SEQUENCE LISTING (20 sequences)

SEQ ID NO: 1 - protein, 822 aa, artificial sequence
  fusion containign E. coli PAP1 and RtcA
MHHHHHHHHHMKVLSREESEAEQAVARPQVTVIPREQHAISRKDISENALKVMYRLNKAGYEAWLVGGGVRDLLLGKKPKDFDVTTNATPEQVRKLFRNCRLVGRRFRLAHVMFGPEIIEVATFRGHHEGNVSDRTTSQRGQNGMLLRDNIFGSIEEDAQRRDFTINSLYYSVADFTVRDYVGGMKDLKDGVIRLIGNPETRYREDPVRMLRAVRFAAKLGMRISPETAEPIPRLATLLNDIPPARLFEESLKLLQAGYGYETYKLLCEYHLFQPLFPTITRYFTENGDSPMERIIEQVLKNTDTRIHNDMRVNPAFLFAAMFWYPLLETAQKIAQESGLTYHDAFALAMNDVLDEACRSLAIPKRLTTLTRDIWQLQLRMSRRQGKRAWKLLEHPKFRAAYDLLALRAEVERNAELQRLVKWWGEFQVSAPPDQKGMLNELDEEPSPRRRTRRPRKRAPRREGTASGSETPGTSESATPESHMMKRMIALDGAQGEGGGQILRSALSLSMITGLPFTITGIRAGRAKPGLLRQHLTAVKAAAEICRATVEGAELGSQRLLFRPGTVRGGDYRFAIGSAGSCTLVLQTVLPALWFADGPSRVEVSGGTDNPSAPPADFIRRVLEPLLAKIGIHQQTTLLRHGFYPAGGGVVATEVSPVTSFNTLQLGERGNIVRLRGEVLLAGVPRHVAEREIATLAASFSLHEQNIHNLPRDQGPGNTVSLEVESENITERFFVVGEKRVSAEVVAAQLVKEVKRYLASPAAVGEYLADQLVLPMALAGAGEFTVAHPSCHLLTNIAVVERFLPVRFGLVEADGVTRVSIE

SEQ ID NO: 2 - protein, 934 aa, artificial sequence
  Fusion of yeast PAP1 and RtcA
MHHHHHHHHHMSSQKVFGITGPVSTVGATAAENKLNDSLIQELKKEGSFETEQETANRVQVLKILQELAQRFVYEVSKKKNMSDGMARDAGGKIFTYGSYRLGVHGPGSDIDTLVVVPKHVTREDFFTVFDSLLRERKELDEIAPVPDAFVPIIKIKFSGISIDLICARLDQPQVPLSLTLSDKNLLRNLDEKDLRALNGTRVTDEILELVPKPNVFRIALRAIKLWAQRRAVYANIFGFPGGVAWAMLVARICQLYPNACSAVILNRFFIILSEWNWPQPVILKPIEDGPLQVRVWNPKIYAQDRSHRMPVITPAYPSMCATHNITESTKKVILQEFVRGVQITNDIFSNKKSWANLFEKNDFFFRYKFYLEITAYTRGSDEQHLKWSGLVESKVRLLVMKLEVLAGIKIAHPFTKPFESSYCCPTEDDYEMIQDKYGSHKTETALNALKLVTDENKEEESIKDAPKAYLSTMYIGLDFNIENKKEKVDIHIPCTEFVNLCRSFNEDYGDHKVFNLALRFVKGYDLPDEVFDENEKRPSKKSKRKNLDARHETVKRSKSDAASGDNINGTTAAVDVNSGSETPGTSESATPESHMMKRMIALDGAQGEGGGQILRSALSLSMITGLPFTITGIRAGRAKPGLLRQHLTAVKAAAEICRATVEGAELGSQRLLFRPGTVRGGDYRFAIGSAGSCTLVLQTVLPALWFADGPSRVEVSGGTDNPSAPPADFIRRVLEPLLAKIGIHQQTTLLRHGFYPAGGGVVATEVSPVTSFNTLQLGERGNIVRLRGEVLLAGVPRHVAEREIATLAASFSLHEQNIHNLPRDQGPGNTVSLEVESENITERFFVVGEKRVSAEVVAAQLVKEVKRYLASPAAVGEYLADQLVLPMALAGAGEFTVAHPSCHLLTNIAVVERFLPVRFGLVEADGVTRVSIE

SEQ ID NO: 3 - DNA, 2469 bp, artificial sequence
  sequence encoding fusion protein
atgcatcatcatcatcatcatcatcatcatatgaaagtgctgagccgcgaagaaagcgaagcggaacaggcggtggcgcgcccgcaggtgaccgtgattccgcgcgaacagcatgcgattagccgcaaagatattagcgaaaacgcgctgaaagtgatgtatcgcctgaacaaagcgggctatgaagcgtggctggtgggcggcggcgtgcgcgatctgctgctgggcaaaaaaccgaaagattttgatgtgaccaccaacgcgaccccggaacaggtgcgcaaactgtttcgcaactgccgcctggtgggccgccgctttcgcctggcgcatgtgatgtttggcccggaaattattgaagtggcgacctttcgcggccatcatgaaggcaacgtgagcgatcgcaccaccagccagcgcggccagaacggcatgctgctgcgcgataacatttttggcagcattgaagaagatgcgcagcgccgcgattttaccattaacagcctgtattatagcgtggcggattttaccgtgcgcgattatgtgggcggcatgaaagatctgaaagatggcgtgattcgcctgattggcaacccggaaacccgctatcgcgaagatccggtgcgcatgctgcgcgcggtgcgctttgcggcgaaactgggcatgcgcattagcccggaaaccgcggaaccgattccgcgcctggcgaccctgctgaacgatattccgccggcgcgcctgtttgaagaaagcctgaaactgctgcaggcgggctatggctatgaaacctataaactgctgtgcgaatatcatctgtttcagccgctgtttccgaccattacccgctattttaccgaaaacggcgatagcccgatggaacgcattattgaacaggtgctgaaaaacaccgatacccgcattcataacgatatgcgcgtgaacccggcgtttctgtttgcggcgatgttttggtatccgctgctggaaaccgcgcagaaaattgcgcaggaaagcggcctgacctatcatgatgcgtttgcgctggcgatgaacgatgtgctggatgaagcgtgccgcagcctggcgattccgaaacgcctgaccaccctgacccgcgatatttggcagctgcagctgcgcatgagccgccgccagggcaaacgcgcgtggaaactgctggaacatccgaaatttcgcgcggcgtatgatctgctggcgctgcgcgcggaagtggaacgcaacgcggaactgcagcgcctggtgaaatggtggggcgaatttcaggtgagcgcgccgccggatcagaaaggcatgctgaacgaactggatgaagaaccgagcccgcgccgccgcacccgccgcccgcgcaaacgcgcgccgcgccgcgaaggcaccgcgagcggcagcgagactcccgggacctcagagtccgccacacccgaaagtcatatgatgaaaaggatgattgcgctggatggcgcacagggcgaaggcggcgggcagatcctgcgctcggcgctgagcctgtcgatgataaccggcctgccatttaccatcaccggcattcgtgccgggcgggcaaaaccgggactgttgcgccagcatctgaccgcggtaaaagcggctgcggaaatttgtagggcaacggtggaaggtgcggagctgggatcgcagcgtctgctcttccggcccggcaccgtgcgcggcggcgattaccgctttgctatcggtagcgccggaagttgtacgctggtgctgcaaacggtgctgcccgcgctgtggtttgccgatggaccttcgcgtgttgaagtgagcggaggcaccgataacccgtcggccccgcctgcggattttatccgccgggtgctggagccgctgctggcgaaaataggaattcatcagcaaaccacgctgttacgtcacggtttttatcctgccggaggcggcgtggtggcaacggaagtctcgccggtgacatcgtttaacaccttgcaacttggcgagcgcgggaacattgtgcggctgcgtggtgaggtgttattagctggcgtaccgcgacatgttgctgagcgtgaaatcgctacgctggcggcaagtttttccctgcatgagcagaatattcataacctgccgcgtgaccaggggccgggtaataccgtttcgcttgaagtcgaaagtgaaaatatcaccgaacgcttttttgtcgtcggtgaaaagcgcgtcagcgccgaggtggtcgcggcacagttggtgaaagaggtgaaacgctacctggcaagcccggcggcggtgggggaatatctcgccgaccagttggtgctaccgatggcgctggcgggcgcgggagaatttacggtcgcccatccctcatgccatctgctgaccaatatcgcggtggtggagcgtttcttgccagtgcggtttggtctggtggaggctgatggcgtaacgcgggtgagcattgaataa

SEQ ID NO: 4 - DNA, 2805 bp, artificial sequenc
  coding sequence for fusion protein
atgcatcatcatcatcatcatcatcatcatatgagctctcaaaaggtttttggtattactggacctgtttccaccgtgggcgccacagcagcagaaaataaattaaatgatagtttaatccaagaactgaaaaaggaaggatcgttcgaaacagagcaagaaactgccaatagggtacaagtgttgaaaatattgcaggaattggcacaaagatttgtttatgaagtatcgaagaagaaaaatatgtcagacgggatggcaagggatgctggtgggaagatttttacgtatgggtcctatagactaggagtccatgggcctggtagtgatatcgatactttggtagttgttccaaaacatgtaactcgggaagatttttttacggtatttgattcactactgagagagaggaaggaactggatgaaattgcacctgtacctgatgcgtttgtcccgattatcaagataaagttcagtggtatttctatcgatttaatctgtgcacgtctagaccaacctcaagtgcctttatccttgactttatcagataaaaatctactgcgaaatctagacgagaaggacttgagagctttgaatggtaccagagtaacagatgagatattagaactggtaccaaagccgaatgttttcagaatcgctttaagagctattaagctatgggcccaaagaagggctgtttatgctaatatttttggttttcctggtggtgtggcttgggccatgctagtggctagaatttgtcaactataccctaacgcctgtagcgcagttatattgaacagatttttcatcattttgtcggaatggaattggccacaacctgttatcttgaaaccaattgaggatggcccgttacaagttcgtgtatggaatccaaagatatatgcccaagacaggtctcatagaatgcccgtcattacaccagcttatccatcaatgtgtgctacccataacatcacggaatctactaaaaaagtcattttacaggaattcgtaagaggcgttcaaattacgaatgatattttttccaataagaagtcctgggccaatttattcgaaaaaaacgattttttctttcgatacaagttctatttagaaattactgcatatacaaggggcagtgacgagcagcatttaaaatggagtggtcttgttgaaagtaaggtaaggcttctagttatgaaactggaggtgttagctggaataaaaattgcacatcctttcaccaaaccctttgaaagtagttattgttgtccaaccgaggatgactatgaaatgattcaagacaaatacggtagtcataaaactgagacagcactgaacgcccttaaactggtaacagatgaaaataaagaggaagaaagtattaaagatgcaccaaaggcatatttaagcaccatgtacataggccttgactttaatattgaaaacaaaaaggaaaaagttgacattcacattccctgcactgaatttgtgaatttatgtcgaagtttcaatgaggattatggtgaccacaaagtattcaatctagccctccgcttcgtaaagggttacgatttgccagatgaagttttcgatgaaaatgaaaagagaccatcaaagaagagtaaaaggaagaatttagatgctagacatgaaaccgtgaagagatctaaatcagatgctgcttcaggtgacaacatcaatggcacaaccgcagctgttgacgtaaacagcggcagcgagactcccgggacctcagagtccgccacacccgaaagtcatatgatgaaaaggatgattgcgctggatggcgcacagggcgaaggcggcgggcagatcctgcgctcggcgctgagcctgtcgatgataaccggcctgccatttaccatcaccggcattcgtgccgggcgggcaaaaccgggactgttgcgccagcatctgaccgcggtaaaagcggctgcggaaatttgtagggcaacggtggaaggtgcggagctgggatcgcagcgtctgctcttccggcccggcaccgtgcgcggcggcgattaccgctttgctatcggtagcgccggaagttgtacgctggtgctgcaaacggtgctgcccgcgctgtggtttgccgatggaccttcgcgtgttgaagtgagcggaggcaccgataacccgtcggccccgcctgcggattttatccgccgggtgctggagccgctgctggcgaaaataggaattcatcagcaaaccacgctgttacgtcacggtttttatcctgccggaggcggcgtggtggcaacggaagtctcgccggtgacatcgtttaacaccttgcaacttggcgagcgcgggaacattgtgcggctgcgtggtgaggtgttattagctggcgtaccgcgacatgttgctgagcgtgaaatcgctacgctggcggcaagtttttccctgcatgagcagaatattcataacctgccgcgtgaccaggggccgggtaataccgtttcgcttgaagtcgaaagtgaaaatatcaccgaacgcttttttgtcgtcggtgaaaagcgcgtcagcgccgaggtggtcgcggcacagttggtgaaagaggtgaaacgctacctggcaagcccggcggcggtgggggaatatctcgccgaccagttggtgctaccgatggcgctggcgggcgcgggagaatttacggtcgcccatccctcatgccatctgctgaccaatatcgcggtggtggagcgtttcttgccagtgcggtttggtctggtggaggctgatggcgtaacgcgggtgagcattgaataa

SEQ ID NO: 5 - DNA, 58 bp, artificial sequence
  biotin primer, second to last n is  C, or G, and the final N is A, C, G, or T
  misc_feature (57)..(58): n is a, c, g, or t
gtgactggagttgacgtgtgctcttccgatctaaaaaaaaaaaaaaaaaaaaaaaann

SEQ ID NO: 6 - DNA, 35 bp, artificial sequence
  adapter sequence, final two nucleotides are rG or rC
  misc_feature (34)..(35): n is a, c, g, t or u
acactctttccctacacgacgctcttccgatctnn

SEQ ID NO: 7 - DNA, 31 bp, artificial sequence
  biotinylated primer
agcgagcgaccaaaggaaccataactgattt

SEQ ID NO: 8 - DNA, 21 bp, artificial sequence
  biotinylated primer
cgaggttatctagagtcacca

SEQ ID NO: 9 - DNA, 22 bp, artificial sequence
  biotinylated primer
tcctagctgcggtatccaggcg

SEQ ID NO: 10 - DNA, 29 bp, artificial sequence
  biotinylated primer
agatagtcaagttcgaccgtcttctcagc

SEQ ID NO: 11 - DNA, 34 bp, artificial sequence
  biotinylated primer
gggcctcgatcagaaggacttgggccccccacga

SEQ ID NO: 12 - DNA, 24 bp, artificial sequence
  biotinylated primer
cgcttggcgccagaagcgagagcc

SEQ ID NO: 13 - DNA, 31 bp, artificial sequence
  biotinylated primer
agcgacgctcagacaggcgtagccccgggag

SEQ ID NO: 14 - DNA, 21 bp, artificial sequence
  biotinylated primer
ccggctatccgaggccaaccg

SEQ ID NO: 15 - DNA, 26 bp, artificial sequence
  biotinylated primer
tgatctgataaatgcacgcatccccc

SEQ ID NO: 16 - DNA, 32 bp, artificial sequence
  biotinylated primer
gtgtcgagggctgactttcaatagatcgcagc

SEQ ID NO: 17 - DNA, 21 bp, artificial sequence
  biotinylated primer
agtagtggtatttcaccggcg

SEQ ID NO: 18 - DNA, 19 bp, artificial sequence
  biotinylated primer
tagaattaccacagttatc

SEQ ID NO: 19 - DNA, 58 bp, artificial sequence
  primer
aatgatacggcgaccaccgagatctacactctttccctacacgacgctcttccgatct

SEQ ID NO: 20 - DNA, 63 bp, artificial sequence
  primer, nnnnnn is a any nucleotide sequenc barcode
  misc_feature (25)..(30): n is a, c, g, or t
caagcagaagacggcatacgagatnnnnnngtgactggagttcagacgtgtgctcttccgatc